European Patent Application EP 4 722 377 A1, published April 8, 2026. Title: Method for production of product. Applicant: FUJIFILM Corporation. The sequence listing filed with the application follows.

SEQUENCE LISTING (4 sequences)

SEQ ID NO: 1 - DNA, 20 bp, synthetic construct
  misc_feature 1..20: note = Description of Artificial Sequence: primer
  source 1..20: mol_type = other DNA
aggtacccaacgccttttct

SEQ ID NO: 2 - DNA, 20 bp, synthetic construct
  misc_feature 1..20: note = Description of Artificial Sequence: primer
  source 1..20: mol_type = other DNA
gaggccagcaagagacaatc

SEQ ID NO: 3 - DNA, 20 bp, synthetic construct
  misc_feature 1..20: note = Description of Artificial Sequence: primer
  source 1..20: mol_type = other DNA
tggtgaagcaggcatctgag

SEQ ID NO: 4 - DNA, 20 bp, synthetic construct
  misc_feature 1..20: note = Description of Artificial Sequence: primer
  source 1..20: mol_type = other DNA
gtccagggtgggcttcttac